European Patent Specification EP 2 524 044 B1, published November 13, 2024. Title: COMPOSITIONS AND METHODS FOR MINIMIZING NORNICOTINE SYNTHESIS IN TOBACCO. Applicant: Dewey, Ralph E. Lewis, Ramsey S. The sequence listing filed with the application follows.

SEQUENCE LISTING (40 sequences)

SEQ ID NO: 1 - DNA, 1551 bp, Nicotiana tabacum
  CDS (1)...(1551): Encodes CYP82E10 nicotine demethylase
atggtttctcccgtagaagccatcgtaggactagtaactcttacacttctcttctacttcatacggaccaaaaaatctcaaaaaccttcaaaaccattaccaccgaaaatccccggagggtggccggtaatcggccatcttttctatttcgatgacgacagcgacgaccgtccattagcacgaaaactcggagacttagctgacaaatacggcccggttttcacttttcggctaggccttccgcttgtgttagttgtaagcagttacgaagctataaaagactgcttctctacaaatgatgccattttctccaatcgtccagcttttctttatggcgaataccttggctacaataatgccatgctatttttgacaaaatacggaccttactggcgaaaaaatagaaaattagtcattcaggaagttctctgtgctagtcgtctcgaaaaattgaagcacgtgagatttggtgaaattcagacgagcattaagaatttatacactcgaattgatggaaattcgagtacgataaatctaaccgattggttagaagaattgaattttggtctgatcgtgaaaatgatcgctgggaaaaattatgaatccggtaaaggagatgaacaagtggagagatttaggaaagcgtttaaggattttataattttatcaatggagtttgtgttatgggatgcttttccaattccattgttcaaatgggtggattttcaaggccatgttaaggccatgaaaaggacatttaaggatatagattctgtttttcagaattggttagaggaacatgtcaagaaaaaagaaaaaatggaggttaatgcagaaggaaatgaacaagatttcattgatgtggtgctttcaaaaatgagtaatgaatatcttgatgaaggctactctcgtgatactgtcataaaagcaacagtgtttagtttagtcttggatgctgcggacacagttgctcttcacatgaattggggaatggcattattgataaacaatcaacatgccttgaagaaagcgcaagaagagatagataaaaaagttggtaaggatagatgggtagaagagagtgatattaaggatttggtatacctccaaactattgttaaagaagtgttacgattatatccaccgggacctttattagtaccccatgaaaatgtagaggattgtgttgttagtggatatcacattcctaaagggactagactattcgcgaacgttatgaaattacagcgcgatcctaaactctggtcaaatcctgataagttcgatccagagagatttttcgctgctgatattgactttcgtggtcaacactatgagtttatcccatttggttctggaagacgatcttgtccggggatgacttatgcaatgcaagtggaacacctaacaatcgcacacttgatccagggtttcaattacaaaactccaaatgacgagcccttggatatgaaggaaggtgcaggattaactatacgtaaggtaaatcctatagaagtggtaattacgcctcgcctgacacctgagctttat

SEQ ID NO: 2 - protein, 517 aa, Nicotiana tabacum
MVSPVEAIVGLVTLTLLFYFIRTKKSQKPSKPLPPKIPGGWPVIGHLFYFDDDSDDRPLARKLGDLADKYGPVFTFRLGLPLVLVVSSYEAIKDCFSTNDAIFSNRPAFLYGEYLGYNNAMLFLTKYGPYWRKNRKLVIQEVLCASRLEKLKHVRFGEIQTSIKNLYTRIDGNSSTINLTDWLEELNFGLIVKMIAGKNYESGKGDEQVERFRKAFKDFIILSMEFVLWDAFPIPLFKWVDFQGHVKAMKRTFKDIDSVFQNWLEEHVKKKEKMEVNAEGNEQDFIDVVLSKMSNEYLDEGYSRDTVIKATVFSLVLDAADTVALHMNWGMALLINNQHALKKAQEEIDKKVGKDRWVEESDIKDLVYLQTIVKEVLRLYPPGPLLVPHENVEDCVVSGYHIPKGTRLFANVMKLQRDPKLWSNPDKFDPERFFAADIDFRGQHYEFIPFGSGRRSCPGMTYAMQVEHLTIAHLIQGFNYKTPNDEPLDMKEGAGLTIRKVNPIEVVITPRLTPELY

SEQ ID NO: 3 - DNA, 818 bp, Nictoiana tabacum
  intron (1)...(818): Intron for CYP82E10 gene
gtaagttcatctcatttttcatttattctttgaggaatagacaggttaatagtaatttaagtaattagattatctaaatactaaggatgagtaaatatggcaaaaatatagaatgataaatggaaaaggatgataattttttatgcccggactaatctaactttgggagttaaagcacttcctaccaatagggacttttcttcaagctcgatcttgatgaaactctgtggttaaaaaaatgagatatanccaattataattgatagaataaaactttattactcccattgagcataacaaaacaaaaaaaagtaaagggacttcttctcttttttagggagaaattctttgattgtttgttaatatagattcatgtttttttttatttctaataataattgtgcttgaatcaggtcgcgctgattcttggctttttagcagcaatagagtcaaagctaatatacatattatttggttttcgaataagttatactgaaattatataatacgggtattaaataataacatgattatttataggatatgctttttttattgggtaaatatattttttttaattaaaaatgaaatatacaagtaaggtataaaacactatttgattttacactagataaatttgccctcgtacatctctaagagaagagctgaaataaatgaattttaaatttcagaaaaaaataaattcattagtataatgagatgtcgatacttgacaattactatactaactagaacaaggttcagcagatagtgacgctaacctatttttgtattgaattattctaatttgtccacag

SEQ ID NO: 4 - DNA, 2636 bp, Nicotiana tabacum
  5'UTR (1)...(114): CYP82E10 5' UTR
  exon (115)...(1053): CYP82E10 exon 1 sequence
  intron (1054)...(1871): CYP82E10 intron sequence
  exon (1872)...(2483): CYP82E10 exon 2 sequence
  3'UTR (2484)...(2636): CYP82E10 3' UTR
ttttcaatttttgttacttttgtatttatcatattattatgcatagccctaaattatctataaaagggaagttggtgatagtttgattcccaagtgcttttctaaaaatccataatggtttctcccgtagaagccatcgtaggactagtaactcttacacttctcttctacttcatacggaccaaaaaatctcaaaaaccttcaaaaccattaccaccgaaaatccccggagggtggccggtaatcggccatcttttctatttcgatgacgacagcgacgaccgtccattagcacgaaaactcggagacttagctgacaaatacggcccggttttcacttttcggctaggccttccgcttgtgttagttgtaagcagttacgaagctataaaagactgcttctctacaaatgatgccattttctccaatcgtccagcttttctttatggcgaataccttggctacaataatgccatgctatttttgacaaaatacggaccttactggcgaaaaaatagaaaattagtcattcaggaagttctctgtgctagtcgtctcgaaaaattgaagcacgtgagatttggtgaaattcagacgagcattaagaatttatacactcgaattgatggaaattcgagtacgataaatctaaccgattggttagaagaattgaattttggtctgatcgtgaaaatgatcgctgggaaaaattatgaatccggtaaaggagatgaacaagtggagagatttaggaaagcgtttaaggattttataattttatcaatggagtttgtgttatgggatgcttttccaattccattgttcaaatgggtggattttcaaggccatgttaaggccatgaaaaggacatttaaggatatagattctgtttttcagaattggttagaggaacatgtcaagaaaaaagaaaaaatggaggttaatgcagaaggaaatgaacaagatttcattgatgtggtgctttcaaaaatgagtaatgaatatcttgatgaaggctactctcgtgatactgtcataaaagcaacagtgtttgtaagttcatctcatttttcatttattctttgaggaatagacaggttaatagtaatttaagtaattagattatctaaatactaaggatgagtaaatatggcaaaaatatagaatgataaatggaaaaggatgataattttttatgcccggactaatctaactttgggagttaaagcacttcctaccaatagggacttttcttcaagctcgatcttgatgaaactctgtggttaaaaaaatgagatatanccaattataattgatagaataaaactttattactcccattgagcataacaaaacaaaaaaaagtaaagggacttcttctcttttttagggagaaattctttgattgtttgttaatatagattcatgtttttttttatttctaataataattgtgcttgaatcaggtcgcgctgattcttggctttttagcagcaatagagtcaaagctaatatacatattatttggttttcgaataagttatactgaaattatataatacgggtattaaataataacatgattatttataggatatgctttttttattgggtaaatatattttttttaattaaaaatgaaatatacaagtaaggtataaaacactatttgattttacactagataaatttgccctcgtacatctctaagagaagagctgaaataaatgaattttaaatttcagaaaaaaataaattcattagtataatgagatgtcgatacttgacaattactatactaactagaacaaggttcagcagatagtgacgctaacctatttttgtattgaattattctaatttgtccacagagtttagtcttggatgctgcggacacagttgctcttcacatgaattggggaatggcattattgataaacaatcaacatgccttgaagaaagcgcaagaagagatagataaaaaagttggtaaggatagatgggtagaagagagtgatattaaggatttggtatacctccaaactattgttaaagaagtgttacgattatatccaccgggacctttattagtaccccatgaaaatgtagaggattgtgttgttagtggatatcacattcctaaagggactagactattcgcgaacgttatgaaattacagcgcgatcctaaactctggtcaaatcctgataagttcgatccagagagatttttcgctgctgatattgactttcgtggtcaacactatgagtttatcccatttggttctggaagacgatcttgtccggggatgacttatgcaatgcaagtggaacacctaacaatcgcacacttgatccagggtttcaattacaaaactccaaatgacgagcccttggatatgaaggaaggtgcaggattaactatacgtaaggtaaatcctatagaagtggtaattacgcctcgcctgacacctgagctttattaaaatctaagatgttttatcttggttgatcattgtttaatactcctagatagatgggtattcatctatctttttaaaattaattgtcagtacgagtgtttctaatttggtaagtttgtaacaacaagtaaagaaggattgtgctagtatgta

SEQ ID NO: 5 - protein, 517 aa, Nicotiana tabacum
  VARIANT (1)...(517): CYP82E10 L148F variant
MVSPVEAIVGLVTLTLLFYFIRTKKSQKPSKPLPPKIPGGWPVIGHLFYFDDDSDDRPLARKLGDLADKYGPVFTFRLGLPLVLVVSSYEAIKDCFSTNDAIFSNRPAFLYGEYLGYNNAMLFLTKYGPYWRKNRKLVIQEVLCASRFEKLKHVRFGEIQTSIKNLYTRIDGNSSTINLTDWLEELNFGLIVKMIAGKNYESGKGDEQVERFRKAFKDFIILSMEFVLWDAFPIPLFKWVDFQGHVKAMKRTFKDIDSVFQNWLEEHVKKKEKMEVNAEGNEQDFIDVVLSKMSNEYLDEGYSRDTVIKATVFSLVLDAADTVALHMNWGMALLINNQHALKKAQEEIDKKVGKDRWVEESDIKDLVYLQTIVKEVLRLYPPGPLLVPHENVEDCVVSGYHIPKGTRLFANVMKLQRDPKLWSNPDKFDPERFFAADIDFRGQHYEFIPFGSGRRSCPGMTYAMQVEHLTIAHLIQGFNYKTPNDEPLDMKEGAGLTIRKVNPIEVVITPRLTPELY

SEQ ID NO: 6 - protein, 517 aa, Nicotiana tabacum
  VARIANT (1)...(517): CYP82E10 G172R Variant
MVSPVEAIVGLVTLTLLFYFIRTKKSQKPSKPLPPKIPGGWPVIGHLFYFDDDSDDRPLARKLGDLADKYGPVFTFRLGLPLVLVVSSYEAIKDCFSTNDAIFSNRPAFLYGEYLGYNNAMLFLTKYGPYWRKNRKLVIQEVLCASRLEKLKHVRFGEIQTSIKNLYTRIDRNSSTINLTDWLEELNFGLIVKMIAGKNYESGKGDEQVERFRKAFKDFIILSMEFVLWDAFPIPLFKWVDFQGHVKAMKRTFKDIDSVFQNWLEEHVKKKEKMEVNAEGNEQDFIDVVLSKMSNEYLDEGYSRDTVIKATVFSLVLDAADTVALHMNWGMALLINNQHALKKAQEEIDKKVGKDRWVEESDIKDLVYLQTIVKEVLRLYPPGPLLVPHENVEDCVVSGYHIPKGTRLFANVMKLQRDPKLWSNPDKFDPERFFAADIDFRGQHYEFIPFGSGRRSCPGMTYAMQVEHLTIAHLIQGFNYKTPNDEPLDMKEGAGLTIRKVNPIEVVITPRLTPELY

SEQ ID NO: 7 - protein, 517 aa, Nicotiana tabacum
  VARIANT (1)...(7): CYP82E10 A344T Variant
MVSPVEAIVGLVTLTLLFYFIRTKKSQKPSKPLPPKIPGGWPVIGHLFYFDDDSDDRPLARKLGDLADKYGPVFTFRLGLPLVLVVSSYEAIKDCFSTNDAIFSNRPAFLYGEYLGYNNAMLFLTKYGPYWRKNRKLVIQEVLCASRLEKLKHVRFGEIQTSIKNLYTRIDGNSSTINLTDWLEELNFGLIVKMIAGKNYESGKGDEQVERFRKAFKDFIILSMEFVLWDAFPIPLFKWVDFQGHVKAMKRTFKDIDSVFQNWLEEHVKKKEKMEVNAEGNEQDFIDVVLSKMSNEYLDEGYSRDTVIKATVFSLVLDAADTVALHMNWGMALLINNQHALKKTQEEIDKKVGKDRWVEESDIKDLVYLQTIVKEVLRLYPPGPLLVPHENVEDCVVSGYHIPKGTRLFANVMKLQRDPKLWSNPDKFDPERFFAADIDFRGQHYEFIPFGSGRRSCPGMTYAMQVEHLTIAHLIQGFNYKTPNDEPLDMKEGAGLTIRKVNPIEVVITPRLTPELY

SEQ ID NO: 8 - protein, 517 aa, Nicotiana tabacum
  VARIANT (1)...(517): CYP82E10 A410T
MVSPVEAIVGLVTLTLLFYFIRTKKSQKPSKPLPPKIPGGWPVIGHLFYFDDDSDDRPLARKLGDLADKYGPVFTFRLGLPLVLVVSSYEAIKDCFSTNDAIFSNRPAFLYGEYLGYNNAMLFLTKYGPYWRKNRKLVIQEVLCASRLEKLKHVRFGEIQTSIKNLYTRIDGNSSTINLTDWLEELNFGLIVKMIAGKNYESGKGDEQVERFRKAFKDFIILSMEFVLWDAFPIPLFKWVDFQGHVKAMKRTFKDIDSVFQNWLEEHVKKKEKMEVNAEGNEQDFIDVVLSKMSNEYLDEGYSRDTVIKATVFSLVLDAADTVALHMNWGMALLINNQHALKKAQEEIDKKVGKDRWVEESDIKDLVYLQTIVKEVLRLYPPGPLLVPHENVEDCVVSGYHIPKGTRLFTNVMKLQRDPKLWSNPDKFDPERFFAADIDFRGQHYEFIPFGSGRRSCPGMTYAMQVEHLTIAHLIQGFNYKTPNDEPLDMKEGAGLTIRKVNPIEVVITPRLTPELY

SEQ ID NO: 9 - protein, 517 aa, Nicotiana tabacum
  VARIANT (1)...(517): CYP82E10 R417H Variant
MVSPVEAIVGLVTLTLLFYFIRTKKSQKPSKPLPPKIPGGWPVIGHLFYFDDDSDDRPLARKLGDLADKYGPVFTFRLGLPLVLVVSSYEAIKDCFSTNDAIFSNRPAFLYGEYLGYNNAMLFLTKYGPYWRKNRKLVIQEVLCASRLEKLKHVRFGEIQTSIKNLYTRIDGNSSTINLTDWLEELNFGLIVKMIAGKNYESGKGDEQVERFRKAFKDFIILSMEFVLWDAFPIPLFKWVDFQGHVKAMKRTFKDIDSVFQNWLEEHVKKKEKMEVNAEGNEQDFIDVVLSKMSNEYLDEGYSRDTVIKATVFSLVLDAADTVALHMNWGMALLINNQHALKKAQEEIDKKVGKDRWVEESDIKDLVYLQTIVKEVLRLYPPGPLLVPHENVEDCVVSGYHIPKGTRLFANVMKLQHDPKLWSNPDKFDPERFFAADIDFRGQHYEFIPFGSGRRSCPGMTYAMQVEHLTIAHLIQGFNYKTPNDEPLDMKEGAGLTIRKVNPIEVVITPRLTPELY

SEQ ID NO: 10 - protein, 517 aa, Nicotiana tabacum
  VARIANT (1)...(517): CYP82E10 P419S Variant
MVSPVEAIVGLVTLTLLFYFIRTKKSQKPSKPLPPKIPGGWPVIGHLFYFDDDSDDRPLARKLGDLADKYGPVFTFRLGLPLVLVVSSYEAIKDCFSTNDAIFSNRPAFLYGEYLGYNNAMLFLTKYGPYWRKNRKLVIQEVLCASRLEKLKHVRFGEIQTSIKNLYTRIDGNSSTINLTDWLEELNFGLIVKMIAGKNYESGKGDEQVERFRKAFKDFIILSMEFVLWDAFPIPLFKWVDFQGHVKAMKRTFKDIDSVFQNWLEEHVKKKEKMEVNAEGNEQDFIDVVLSKMSNEYLDEGYSRDTVIKATVFSLVLDAADTVALHMNWGMALLINNQHALKKAQEEIDKKVGKDRWVEESDIKDLVYLQTIVKEVLRLYPPGPLLVPHENVEDCVVSGYHIPKGTRLFANVMKLQRDSKLWSNPDKFDPERFFAADIDFRGQHYEFIPFGSGRRSCPGMTYAMQVEHLTIAHLIQGFNYKTPNDEPLDMKEGAGLTIRKVNPIEVVITPRLTPELY

SEQ ID NO: 11 - protein, 517 aa, Nicotiana tabacum
  VARIANT (1)...(517): CYP82E10 G79S Variant
MVSPVEAIVGLVTLTLLFYFIRTKKSQKPSKPLPPKIPGGWPVIGHLFYFDDDSDDRPLARKLGDLADKYGPVFTFRLSLPLVLVVSSYEAIKDCFSTNDAIFSNRPAFLYGEYLGYNNAMLFLTKYGPYWRKNRKLVIQEVLCASRLEKLKHVRFGEIQTSIKNLYTRIDGNSSTINLTDWLEELNFGLIVKMIAGKNYESGKGDEQVERFRKAFKDFIILSMEFVLWDAFPIPLFKWVDFQGHVKAMKRTFKDIDSVFQNWLEEHVKKKEKMEVNAEGNEQDFIDVVLSKMSNEYLDEGYSRDTVIKATVFSLVLDAADTVALHMNWGMALLINNQHALKKAQEEIDKKVGKDRWVEESDIKDLVYLQTIVKEVLRLYPPGPLLVPHENVEDCVVSGYHIPKGTRLFANVMKLQRDPKLWSNPDKFDPERFFAADIDFRGQHYEFIPFGSGRRSCPGMTYAMQVEHLTIAHLIQGFNYKTPNDEPLDMKEGAGLTIRKVNPIEVVITPRLTPELY

SEQ ID NO: 12 - protein, 517 aa, Nicotiana tabacum
  VARIANT (1)...(517): CYP82E10 P107S Variant
MVSPVEAIVGLVTLTLLFYFIRTKKSQKPSKPLPPKIPGGWPVIGHLFYFDDDSDDRPLARKLGDLADKYGPVFTFRLGLPLVLVVSSYEAIKDCFSTNDAIFSNRSAFLYGEYLGYNNAMLFLTKYGPYWRKNRKLVIQEVLCASRLEKLKHVRFGEIQTSIKNLYTRIDGNSSTINLTDWLEELNFGLIVKMIAGKNYESGKGDEQVERFRKAFKDFIILSMEFVLWDAFPIPLFKWVDFQGHVKAMKRTFKDIDSVFQNWLEEHVKKKEKMEVNAEGNEQDFIDVVLSKMSNEYLDEGYSRDTVIKATVFSLVLDAADTVALHMNWGMALLINNQHALKKAQEEIDKKVGKDRWVEESDIKDLVYLQTIVKEVLRLYPPGPLLVPHENVEDCVVSGYHIPKGTRLFANVMKLQRDPKLWSNPDKFDPERFFAADIDFRGQHYEFIPFGSGRRSCPGMTYAMQVEHLTIAHLIQGFNYKTPNDEPLDMKEGAGLTIRKVNPIEVVITPRLTPELY

SEQ ID NO: 13 - protein, 517 aa, Nicotiana tabacum
  VARIANT (1)...(517): CYP82E10 P382S Variant
MVSPVEAIVGLVTLTLLFYFIRTKKSQKPSKPLPPKIPGGWPVIGHLFYFDDDSDDRPLARKLGDLADKYGPVFTFRLGLPLVLVVSSYEAIKDCFSTNDAIFSNRPAFLYGEYLGYNNAMLFLTKYGPYWRKNRKLVIQEVLCASRLEKLKHVRFGEIQTSIKNLYTRIDGNSSTINLTDWLEELNFGLIVKMIAGKNYESGKGDEQVERFRKAFKDFIILSMEFVLWDAFPIPLFKWVDFQGHVKAMKRTFKDIDSVFQNWLEEHVKKKEKMEVNAEGNEQDFIDVVLSKMSNEYLDEGYSRDTVIKATVFSLVLDAADTVALHMNWGMALLINNQHALKKAQEEIDKKVGKDRWVEESDIKDLVYLQTIVKEVLRLYPSGPLLVPHENVEDCVVSGYHIPKGTRLFANVMKLQRDPKLWSNPDKFDPERFFAADIDFRGQHYEFIPFGSGRRSCPGMTYAMQVEHLTIAHLIQGFNYKTPNDEPLDMKEGAGLTIRKVNPIEVVITPRLTPELY

SEQ ID NO: 14 - protein, 517 aa, Nicotiana tabacum
MLSPIEAIVGLVTFTFLFFFLWTKKSQKPSKPLPPKIPGGWPVIGHLFHFNDDGDDRPLARKLGDLADKYGPVFTFRLGLPLVLVVSSYEAVKDCFSTNDAIFSNRPAFLYGDYLGYNNAMLFLANYGPYWRKNRKLVIQEVLSASRLEKFKHVRFARIQASIKNLYTRIDGNSSTINLTDWLEELNFGLIVKMIAGKNYESGKGDEQVERFKKAFKDFMILSMEFVLWDAFPIPLFKWVDFQGHVKAMKRTFKDIDSVFQNWLEEHINKREKMEVNAEGNEQDFIDVVLSKMSNEYLGEGYSRDTVIKATVFSLVLDAADTVALHINWGMALLINNQKALTKAQEEIDTKVGKDRWVEESDIKDLVYLQAIVKEVLRLYPPGPLLVPHENVEDCVVSGYHIPKGTRLFANVMKLQRDPKLWSDPDTFDPERFIATDIDFRGQYYKYIPFGSGRRSCPRMTYALQVEHLTMAHLIQGFNYRTPNDEPLDMKEGAGITIRKVNPVELIIAPRLAPELY

SEQ ID NO: 15 - protein, 517 aa, Nicotiana tabacum
  VARIANT (1)...(517): CYP82E4 P38L Variant
MLSPIEAIVGLVTFTFLFFFLWTKKSQKPSKPLPPKILGGWPVIGHLFHFNDDGDDRPLARKLGDLADKYGPVFTFRLGLPLVLVVSSYEAVKDCFSTNDAIFSNRPAFLYGDYLGYNNAMLFLANYGPYWRKNRKLVIQEVLSASRLEKFKHVRFARIQASIKNLYTRIDGNSSTINLTDWLEELNFGLIVKMIAGKNYESGKGDEQVERFKKAFKDFMILSMEFVLWDAFPIPLFKWVDFQGHVKAMKRTFKDIDSVFQNWLEEHINKREKMEVNAEGNEQDFIDVVLSKMSNEYLGEGYSRDTVIKATVFSLVLDAADTVALHINWGMALLINNQKALTKAQEEIDTKVGKDRWVEESDIKDLVYLQAIVKEVLRLYPPGPLLVPHENVEDCVVSGYHIPKGTRLFANVMKLQRDPKLWSDPDTFDPERFIATDIDFRGQYYKYIPFGSGRRSCPGMTYALQVEHLTMAHLIQGFNYRTPNDEPLDMKEGAGITIRKVNPVELIIAPRLAPELY

SEQ ID NO: 16 - protein, 517 aa, Nicotiana tabacum
  VARIANT (1)...(517): CYP82E4 D171N Variant
MLSPIEAIVGLVTFTFLFFFLWTKKSQKPSKPLPPKIPGGWPVIGHLFHFNDDGDDRPLARKLGDLADKYGPVFTFRLGLPLVLVVSSYEAVKDCFSTNDAIFSNRPAFLYGDYLGYNNAMLFLANYGPYWRKNRKLVIQEVLSASRLEKFKHVRFARIQASIKNLYTRINGNSSTINLTDWLEELNFGLIVKMIAGKNYESGKGDEQVERFKKAFKDFMILSMEFVLWDAFPIPLFKWVDFQGHVKAMKRTFKDIDSVFQNWLEEHINKREKMEVNAEGNEQDFIDVVLSKMSNEYLGEGYSRDTVIKATVFSLVLDAADTVALHINWGMALLINNQKALTKAQEEIDTKVGKDRWVEESDIKDLVYLQAIVKEVLRLYPPGPLLVPHENVEDCVVSGYHIPKGTRLFANVMKLQRDPKLWSDPDTFDPERFIATDIDFRGQYYKYIPFGSGRRSCPGMTYALQVEHLTMAHLIQGFNYRTPNDEPLDMKEGAGITIRKVNPVELIIAPRLAPELY

SEQ ID NO: 17 - protein, 517 aa, Nicotiana tabacum
  VARIANT (1)...(517): CYP82E4 E201K Variant
MLSPIEAIVGLVTFTFLFFFLWTKKSQKPSKPLPPKIPGGWPVIGHLFHFNDDGDDRPLARKLGDLADKYGPVFTFRLGLPLVLVVSSYEAVKDCFSTNDAIFSNRPAFLYGDYLGYNNAMLFLANYGPYWRKNRKLVIQEVLSASRLEKFKHVRFARIQASIKNLYTRIDGNSSTINLTDWLEELNFGLIVKMIAGKNYKSGKGDEQVERFKKAFKDFMILSMEFVLWDAFPIPLFKWVDFQGHVKAMKRTFKDIDSVFQNWLEEHINKREKMEVNAEGNEQDFIDVVLSKMSNEYLGEGYSRDTVIKATVFSLVLDAADTVALHINWGMALLINNQKALTKAQEEIDTKVGKDRWVEESDIKDLVYLQAIVKEVLRLYPPGPLLVPHENVEDCVVSGYHIPKGTRLFANVMKLQRDPKLWSDPDTFDPERFIATDIDFRGQYYKYIPFGSGRRSCPGMTYALQVEHLTMAHLIQGFNYRTPNDEPLDMKEGAGITIRKVNPVELIIAPRLAPELY

SEQ ID NO: 18 - protein, 517 aa, Nicotiana tabacum
  VARIANT (1)...(517): CYP82E4 R169Q Variant
MLSPIEAIVGLVTFTFLFFFLWTKKSQKPSKPLPPKIPGGWPVIGHLFHFNDDGDDRPLARKLGDLADKYGPVFTFRLGLPLVLVVSSYEAVKDCFSTNDAIFSNRPAFLYGDYLGYNNAMLFLANYGPYWRKNRKLVIQEVLSASRLEKFKHVRFARIQASIKNLYTQIDGNSSTINLTDWLEELNFGLIVKMIAGKNYESGKGDEQVERFKKAFKDFMILSMEFVLWDAFPIPLFKWVDFQGHVKAMKRTFKDIDSVFQNWLEEHINKREKMEVNAEGNEQDFIDVVLSKMSNEYLGEGYSRDTVIKATVFSLVLDAADTVALHINWGMALLINNQKALTKAQEEIDTKVGKDRWVEESDIKDLVYLQAIVKEVLRLYPPGPLLVPHENVEDCVVSGYHIPKGTRLFANVMKLQRDPKLWSDPDTFDPERFIATDIDFRGQYYKYIPFGSGRRSCPGMTYALQVEHLTMAHLIQGFNYRTPNDEPLDMKEGAGITIRKVNPVELIIAPRLAPELY

SEQ ID NO: 19 - protein, 517 aa, Nicotiana tabacum; identical to SEQ ID NO: 14
  VARIANT (1)...(517): CYP82E4 G459R Variant

SEQ ID NO: 20 - protein, 517 aa, Nicotiana tabacum
  VARIANT (1)...(517): CYP82E4 T427I Variant
MLSPIEAIVGLVTFTFLFFFLWTKKSQKPSKPLPPKIPGGWPVIGHLFHFNDDGDDRPLARKLGDLADKYGPVFTFRLGLPLVLVVSSYEAVKDCFSTNDAIFSNRPAFLYGDYLGYNNAMLFLANYGPYWRKNRKLVIQEVLSASRLEKFKHVRFARIQASIKNLYTRIDGNSSTINLTDWLEELNFGLIVKMIAGKNYESGKGDEQVERFKKAFKDFMILSMEFVLWDAFPIPLFKWVDFQGHVKAMKRTFKDIDSVFQNWLEEHINKREKMEVNAEGNEQDFIDVVLSKMSNEYLGEGYSRDTVIKATVFSLVLDAADTVALHINWGMALLINNQKALTKAQEEIDTKVGKDRWVEESDIKDLVYLQAIVKEVLRLYPPGPLLVPHENVEDCVVSGYHIPKGTRLFANVMKLQRDPKLWSDPDIFDPERFIATDIDFRGQYYKYIPFGSGRRSCPGMTYALQVEHLTMAHLIQGFNYRTPNDEPLDMKEGAGITIRKVNPVELIIAPRLAPELY

SEQ ID NO: 21 - protein, 517 aa, Nicotiana tabacum
  VARIANT (1)...(517): CYP82E4 V376M Variant
MLSPIEAIVGLVTFTFLFFFLWTKKSQKPSKPLPPKIPGGWPVIGHLFHFNDDGDDRPLARKLGDLADKYGPVFTFRLGLPLVLVVSSYEAVKDCFSTNDAIFSNRPAFLYGDYLGYNNAMLFLANYGPYWRKNRKLVIQEVLSASRLEKFKHVRFARIQASIKNLYTRIDGNSSTINLTDWLEELNFGLIVKMIAGKNYESGKGDEQVERFKKAFKDFMILSMEFVLWDAFPIPLFKWVDFQGHVKAMKRTFKDIDSVFQNWLEEHINKREKMEVNAEGNEQDFIDVVLSKMSNEYLGEGYSRDTVIKATVFSLVLDAADTVALHINWGMALLINNQKALTKAQEEIDTKVGKDRWVEESDIKDLVYLQAIVKEMLRLYPPGPLLVPHENVEDCVVSGYHIPKGTRLFANVMKLQRDPKLWSDPDTFDPERFIATDIDFRGQYYKYIPFGSGRRSCPGMTYALQVEHLTMAHLIQGFNYRTPNDEPLDMKEGAGITIRKVNPVELIIAPRLAPELY

SEQ ID NO: 22 - protein, 328 aa, Nicotiana tabacum
  VARIANT (1)...(328): CYP82E4 W329Stop Variant
MLSPIEAIVGLVTFTFLFFFLWTKKSQKPSKPLPPKIPGGWPVIGHLFHFNDDGDDRPLARKLGDLADKYGPVFTFRLGLPLVLVVSSYEAVKDCFSTNDAIFSNRPAFLYGDYLGYNNAMLFLANYGPYWRKNRKLVIQEVLSASRLEKFKHVRFARIQASIKNLYTRIDGNSSTINLTDWLEELNFGLIVKMIAGKNYESGKGDEQVERFKKAFKDFMILSMEFVLWDAFPIPLFKWVDFQGHVKAMKRTFKDIDSVFQNWLEEHINKREKMEVNAEGNEQDFIDVVLSKMSNEYLGEGYSRDTVIKATVFSLVLDAADTVALHIN

SEQ ID NO: 23 - protein, 517 aa, Nicotiana tabacum
  VARIANT (1)...(517): CYP82E4 K364N Variant
MLSPIEAIVGLVTFTFLFFFLWTKKSQKPSKPLPPKIPGGWPVIGHLFHFNDDGDDRPLARKLGDLADKYGPVFTFRLGLPLVLVVSSYEAVKDCFSTNDAIFSNRPAFLYGDYLGYNNAMLFLANYGPYWRKNRKLVIQEVLSASRLEKFKHVRFARIQASIKNLYTRIDGNSSTINLTDWLEELNFGLIVKMIAGKNYESGKGDEQVERFKKAFKDFMILSMEFVLWDAFPIPLFKWVDFQGHVKAMKRTFKDIDSVFQNWLEEHINKREKMEVNAEGNEQDFIDVVLSKMSNEYLGEGYSRDTVIKATVFSLVLDAADTVALHINWGMALLINNQKALTKAQEEIDTKVGKDRWVEESDINDLVYLQAIVKEVLRLYPPGPLLVPHENVEDCVVSGYHIPKGTRLFANVMKLQRDPKLWSDPDTFDPERFIATDIDFRGQYYKYIPFGSGRRSCPGMTYALQVEHLTMAHLIQGFNYRTPNDEPLDMKEGAGITIRKVNPVELIIAPRLAPELY

SEQ ID NO: 24 - protein, 517 aa, Nicotiana tabacum
  VARIANT (1)...(517): CYP82E4 P382S Variant
MLSPIEAIVGLVTFTFLFFFLWTKKSQKPSKPLPPKIPGGWPVIGHLFHFNDDGDDRPLARKLGDLADKYGPVFTFRLGLPLVLVVSSYEAVKDCFSTNDAIFSNRPAFLYGDYLGYNNAMLFLANYGPYWRKNRKLVIQEVLSASRLEKFKHVRFARIQASIKNLYTRIDGNSSTINLTDWLEELNFGLIVKMIAGKNYESGKGDEQVERFKKAFKDFMILSMEFVLWDAFPIPLFKWVDFQGHVKAMKRTFKDIDSVFQNWLEEHINKREKMEVNAEGNEQDFIDVVLSKMSNEYLGEGYSRDTVIKATVFSLVLDAADTVALHINWGMALLINNQKALTKAQEEIDTKVGKDRWVEESDIKDLVYLQAIVKEVLRLYPSGPLLVPHENVEDCVVSGYHIPKGTRLFANVMKLQRDPKLWSDPDTFDPERFIATDIDFRGQYYKYIPFGSGRRSCPGMTYALQVEHLTMAHLIQGFNYRTPNDEPLDMKEGAGITIRKVNPVELIIAPRLAPELY

SEQ ID NO: 25 - protein, 517 aa, Nicotiana tabacum
  VARIANT (1)...(517): CYP82E4 P458S Variant
MLSPIEAIVGLVTFTFLFFFLWTKKSQKPSKPLPPKIPGGWPVIGHLFHFNDDGDDRPLARKLGDLADKYGPVFTFRLGLPLVLVVSSYEAVKDCFSTNDAIFSNRPAFLYGDYLGYNNAMLFLANYGPYWRKNRKLVIQEVLSASRLEKFKHVRFARIQASIKNLYTRIDGNSSTINLTDWLEELNFGLIVKMIAGKNYESGKGDEQVERFKKAFKDFMILSMEFVLWDAFPIPLFKWVDFQGHVKAMKRTFKDIDSVFQNWLEEHINKREKMEVNAEGNEQDFIDVVLSKMSNEYLGEGYSRDTVIKATVFSLVLDAADTVALHINWGMALLINNQKALTKAQEEIDTKVGKDRWVEESDIKDLVYLQAIVKEVLRLYPPGPLLVPHENVEDCVVSGYHIPKGTRLFANVMKLQRDPKLWSDPDTFDPERFIATDIDFRGQYYKYIPFGSGRRSCSGMTYALQVEHLTMAHLIQGFNYRTPNDEPLDMKEGAGITIRKVNPVELIIAPRLAPELY

SEQ ID NO: 26 - protein, 517 aa, Nicotiana tabacum
MVSPVEAIVGLVTLTLLFYFLWPKKFQIPSKPLPPKIPGGWPVIGHLFYFDDDGDDRPLARKLGDLADKYGPVFTFRLGLPLVLVVSSYEAVKDCFSTNDAIFSNRPAFLYGEYLGYSNAMLFLTKYGPYWRKNRKLVIQEVLSASRLEKLKHVRFGKIQTSIKSLYTRIDGNSSTINLTDWLEELNFGLIVKMIAGKNYESGKGDEQVERFRKAFKDFIILSMEFVLWDAFPIPLFKWVDFQGHVKAMKRTFKDIDSVFQNWLEEHVKKREKMEVNAQGNEQDFIDVVLSKMSNEYLDEGYSRDTVIKATVFSLVLDAADTVALHMNWGMALLINNQHALKKAQEEIDKKVGKERWVEESDIKDLVYLQAIVKEVLRLYPPGPLLVPHENVEDCVVSGYHIPKGTRLFANVMKLQRDPKLWSNPDKFDPERFFADDIDYRGQHYEFIPFGSGRRSCPGMTYALQAEHLTIAHLIQGFNYKTPNDEPLDMKEGAGLTIRKVNPVEVTITARLAPELY

SEQ ID NO: 27 - protein, 517 aa, Nicotiana tabacum
  VARIANT (1)...(517): CYP82E5 P72L Variant
MVSPVEAIVGLVTLTLLFYFLWPKKFQIPSKPLPPKIPGGWPVIGHLFYFDDDGDDRPLARKLGDLADKYGLVFTFRLGLPLVLVVSSYEAVKDCFSTNDAIFSNRPAFLYGEYLGYSNAMLFLTKYGPYWRKNRKLVIQEVLSASRLEKLKHVRFGKIQTSIKSLYTRIDGNSSTINLTDWLEELNFGLIVKMIAGKNYESGKGDEQVERFRKAFKDFIILSMEFVLWDAFPIPLFKWVDFQGHVKAMKRTFKDIDSVFQNWLEEHVKKREKMEVNAQGNEQDFIDVVLSKMSNEYLDEGYSRDTVIKATVFSLVLDAADTVALHMNWGMALLINNQHALKKAQEEIDKKVGKERWVEESDIKDLVYLQAIVKEVLRLYPPGPLLVPHENVEDCVVSGYHIPKGTRLFANVMKLQRDPKLWSNPDKFDPERFFADDIDYRGQHYEFIPFGSGRRSCPGMTYALQAEHLTIAHLIQGFNYKTPNDEPLDMKEGAGLTIRKVNPVEVTITARLAPELY

SEQ ID NO: 28 - protein, 517 aa, Nicotiana tabacum
  VARIANT (1)...(517): CYP82E5 L143F Variant
MVSPVEAIVGLVTLTLLFYFLWPKKFQIPSKPLPPKIPGGWPVIGHLFYFDDDGDDRPLARKLGDLADKYGPVFTFRLGLPLVLVVSSYEAVKDCFSTNDAIFSNRPAFLYGEYLGYSNAMLFLTKYGPYWRKNRKLVIQEVFSASRLEKLKHVRFGKIQTSIKSLYTRIDGNSSTINLTDWLEELNFGLIVKMIAGKNYESGKGDEQVERFRKAFKDFIILSMEFVLWDAFPIPLFKWVDFQGHVKAMKRTFKDIDSVFQNWLEEHVKKREKMEVNAQGNEQDFIDVVLSKMSNEYLDEGYSRDTVIKATVFSLVLDAADTVALHMNWGMALLINNQHALKKAQEEIDKKVGKERWVEESDIKDLVYLQAIVKEVLRLYPPGPLLVPHENVEDCVVSGYHIPKGTRLFANVMKLQRDPKLWSNPDKFDPERFFADDIDYRGQHYEFIPFGSGRRSCPGMTYALQAEHLTIAHLIQGFNYKTPNDEPLDMKEGAGLTIRKVNPVEVTITARLAPELY

SEQ ID NO: 29 - protein, 517 aa, Nicotiana tabacum
  VARIANT (1)...(517): CYP82E5 S174L Variant
MVSPVEAIVGLVTLTLLFYFLWPKKFQIPSKPLPPKIPGGWPVIGHLFYFDDDGDDRPLARKLGDLADKYGPVFTFRLGLPLVLVVSSYEAVKDCFSTNDAIFSNRPAFLYGEYLGYSNAMLFLTKYGPYWRKNRKLVIQEVLSASRLEKLKHVRFGKIQTSIKSLYTRIDGNLSTINLTDWLEELNFGLIVKMIAGKNYESGKGDEQVERFRKAFKDFIILSMEFVLWDAFPIPLFKWVDFQGHVKAMKRTFKDIDSVFQNWLEEHVKKREKMEVNAQGNEQDFIDVVLSKMSNEYLDEGYSRDTVIKATVFSLVLDAADTVALHMNWGMALLINNQHALKKAQEEIDKKVGKERWVEESDIKDLVYLQAIVKEVLRLYPPGPLLVPHENVEDCVVSGYHIPKGTRLFANVMKLQRDPKLWSNPDKFDPERFFADDIDYRGQHYEFIPFGSGRRSCPGMTYALQAEHLTIAHLIQGFNYKTPNDEPLDMKEGAGLTIRKVNPVEVTITARLAPELY

SEQ ID NO: 30 - protein, 517 aa, Nicotiana tabacum
  VARIANT (1)...(517): CYP82E5 M224I  Variant
MVSPVEAIVGLVTLTLLFYFLWPKKFQIPSKPLPPKIPGGWPVIGHLFYFDDDGDDRPLARKLGDLADKYGPVFTFRLGLPLVLVVSSYEAVKDCFSTNDAIFSNRPAFLYGEYLGYSNAMLFLTKYGPYWRKNRKLVIQEVLSASRLEKLKHVRFGKIQTSIKSLYTRIDGNSSTINLTDWLEELNFGLIVKMIAGKNYESGKGDEQVERFRKAFKDFIILSIEFVLWDAFPIPLFKWVDFQGHVKAMKRTFKDIDSVFQNWLEEHVKKREKMEVNAQGNEQDFIDVVLSKMSNEYLDEGYSRDTVIKATVFSLVLDAADTVALHMNWGMALLINNQHALKKAQEEIDKKVGKERWVEESDIKDLVYLQAIVKEVLRLYPPGPLLVPHENVEDCVVSGYHIPKGTRLFANVMKLQRDPKLWSNPDKFDPERFFADDIDYRGQHYEFIPFGSGRRSCPGMTYALQAEHLTIAHLIQGFNYKTPNDEPLDMKEGAGLTIRKVNPVEVTITARLAPELY

SEQ ID NO: 31 - protein, 517 aa, Nicotiana tabacum
  VARIANT (1)...(517): CYP82E5 P235S Variant
MVSPVEAIVGLVTLTLLFYFLWPKKFQIPSKPLPPKIPGGWPVIGHLFYFDDDGDDRPLARKLGDLADKYGPVFTFRLGLPLVLVVSSYEAVKDCFSTNDAIFSNRPAFLYGEYLGYSNAMLFLTKYGPYWRKNRKLVIQEVLSASRLEKLKHVRFGKIQTSIKSLYTRIDGNSSTINLTDWLEELNFGLIVKMIAGKNYESGKGDEQVERFRKAFKDFIILSMEFVLWDAFPISLFKWVDFQGHVKAMKRTFKDIDSVFQNWLEEHVKKREKMEVNAQGNEQDFIDVVLSKMSNEYLDEGYSRDTVIKATVFSLVLDAADTVALHMNWGMALLINNQHALKKAQEEIDKKVGKERWVEESDIKDLVYLQAIVKEVLRLYPPGPLLVPHENVEDCVVSGYHIPKGTRLFANVMKLQRDPKLWSNPDKFDPERFFADDIDYRGQHYEFIPFGSGRRSCPGMTYALQAEHLTIAHLIQGFNYKTPNDEPLDMKEGAGLTIRKVNPVEVTITARLAPELY

SEQ ID NO: 32 - protein, 517 aa, Nicotiana tabacum
  VARIANT (1)...(517): CYP82E5 A410V Variant
MVSPVEAIVGLVTLTLLFYFLWPKKFQIPSKPLPPKIPGGWPVIGHLFYFDDDGDDRPLARKLGDLADKYGPVFTFRLGLPLVLVVSSYEAVKDCFSTNDAIFSNRPAFLYGEYLGYSNAMLFLTKYGPYWRKNRKLVIQEVLSASRLEKLKHVRFGKIQTSIKSLYTRIDGNSSTINLTDWLEELNFGLIVKMIAGKNYESGKGDEQVERFRKAFKDFIILSMEFVLWDAFPIPLFKWVDFQGHVKAMKRTFKDIDSVFQNWLEEHVKKREKMEVNAQGNEQDFIDVVLSKMSNEYLDEGYSRDTVIKATVFSLVLDAADTVALHMNWGMALLINNQHALKKAQEEIDKKVGKERWVEESDIKDLVYLQAIVKEVLRLYPPGPLLVPHENVEDCVVSGYHIPKGTRLFVNVMKLQRDPKLWSNPDKFDPERFFADDIDYRGQHYEFIPFGSGRRSCPGMTYALQAEHLTIAHLIQGFNYKTPNDEPLDMKEGAGLTIRKVNPVEVTITARLAPELY

SEQ ID NO: 33 - protein, 421 aa, Nicotiana tabacum
  VARIANT (1)...(421): CYP82E5 W422Stop Variant
MVSPVEAIVGLVTLTLLFYFLWPKKFQIPSKPLPPKIPGGWPVIGHLFYFDDDGDDRPLARKLGDLADKYGPVFTFRLGLPLVLVVSSYEAVKDCFSTNDAIFSNRPAFLYGEYLGYSNAMLFLTKYGPYWRKNRKLVIQEVLSASRLEKLKHVRFGKIQTSIKSLYTRIDGNSSTINLTDWLEELNFGLIVKMIAGKNYESGKGDEQVERFRKAFKDFIILSMEFVLWDAFPIPLFKWVDFQGHVKAMKRTFKDIDSVFQNWLEEHVKKREKMEVNAQGNEQDFIDVVLSKMSNEYLDEGYSRDTVIKATVFSLVLDAADTVALHMNWGMALLINNQHALKKAQEEIDKKVGKERWVEESDIKDLVYLQAIVKEVLRLYPPGPLLVPHENVEDCVVSGYHIPKGTRLFANVMKLQRDPKL

SEQ ID NO: 34 - protein, 517 aa, Nicotiana tabacum
  VARIANT (1)...(517): CYP82E5 P449L
MVSPVEAIVGLVTLTLLFYFLWPKKFQIPSKPLPPKIPGGWPVIGHLFYFDDDGDDRPLARKLGDLADKYGPVFTFRLGLPLVLVVSSYEAVKDCFSTNDAIFSNRPAFLYGEYLGYSNAMLFLTKYGPYWRKNRKLVIQEVLSASRLEKLKHVRFGKIQTSIKSLYTRIDGNSSTINLTDWLEELNFGLIVKMIAGKNYESGKGDEQVERFRKAFKDFIILSMEFVLWDAFPIPLFKWVDFQGHVKAMKRTFKDIDSVFQNWLEEHVKKREKMEVNAQGNEQDFIDVVLSKMSNEYLDEGYSRDTVIKATVFSLVLDAADTVALHMNWGMALLINNQHALKKAQEEIDKKVGKERWVEESDIKDLVYLQAIVKEVLRLYPPGPLLVPHENVEDCVVSGYHIPKGTRLFANVMKLQRDPKLWSNPDKFDPERFFADDIDYRGQHYEFILFGSGRRSCPGMTYALQAEHLTIAHLIQGFNYKTPNDEPLDMKEGAGLTIRKVNPVEVTITARLAPELY

SEQ ID NO: 35 - DNA, 23 bp, Artificial Sequence
  forward primer for exon 1 of CYP82E10 gene
gtgatagtttgattcccaagtgc

SEQ ID NO: 36 - DNA, 22 bp, Artificial Sequence
  reverse primer for exon 1 of CYP82E10 gene
ctcccaaagttagattagtccg

SEQ ID NO: 37 - DNA, 18 bp, Artificial Sequence
  forward primer for exon 2 of CYP82E10 gene
aggtcgcgctgattcttg

SEQ ID NO: 38 - DNA, 26 bp, Artificial Sequence
  reverse primer for exon 2 of CYP82E10 gene
agatgaatacccatctatctaggagt

SEQ ID NO: 39 - DNA, 2752 bp, Nicotiana tabacum
  5'UTR (1)...(50): CYP82E4v2 5' UTR
  exon (51)...(989): CYP82E4v2 exon 1 sequence
  intron (990)...(1990): CYP82E4v2 intron sequence
  exon (1991)...(2602): CYP82E4v2 exon 2 sequence
  3'UTR (2603)...(2685): CYP82E4v2 3' UTR
aaggaagttgccgatagttatattctcaacttcttatctaaaaatccataatgctttctcccatagaagccattgtaggactagtaaccttcacatttctcttcttcttcctatggacaaaaaaatctcaaaaaccttcaaaacccttaccaccgaaaatccccggaggatggccggtaatcggccatcttttccacttcaatgacgacggcgacgaccgtccattagctcgaaaactcggagacttagctgacaaatacggccccgttttcacttttcggctaggccttccccttgtcttagttgtaagcagttacgaagctgtaaaagactgtttctctacaaatgacgccattttttccaatcgtccagcttttctttacggcgattaccttggctacaataatgccatgctatttttggccaattacggaccttactggcgaaaaaatcgaaaattagttattcaggaagttctctccgctagtcgtctcgaaaaattcaaacacgtgagatttgcaagaattcaagcgagcattaagaatttatatactcgaattgatggaaattcgagtacgataaatttaactgattggttagaagaattgaattttggtctgatcgtgaagatgatcgctggaaaaaattatgaatccggtaaaggagatgaacaagtggagagatttaagaaagcgtttaaggattttatgattttatcaatggagtttgtgttatgggatgcatttccaattccattatttaaatgggtggattttcaagggcatgttaaggctatgaaaaggacttttaaagatatagattctgtttttcagaattggttagaggaacatattaataaaagagaaaaaatggaggttaatgcagaagggaatgaacaagatttcattgatgtggtgctttcaaaaatgagtaatgaatatcttggtgaaggttactctcgtgatactgtcattaaagcaacggtgtttgtaagttcatctgtcatttttcatttattcacttttattttgaggagcagacatgttaataataatttggagcaactgtaaagttatctatgtgtacaggttcgagcctcaggtgcaaccactaatgcttgtattagattatgttgtctgcatcatacccctaattggagtgtggctcttcccgaaccctgcaatgctggatgctggatgctttatgtatcagactgacctttttgttaaactatctaaatactaaggatgatgatttaataaaaatatagaatggtaaacagaaaaagatgagattatttttggggctatatggattcgcccgggctttgggaggtaaaacggtatctaccagttgagactttactccagaactttatctcgagagctctgaataaaaatgaaatagtatttaccactccaaaatctttgatggtaaaaagatgagatataacctcttataattgattgaaccacgttgatagaataaaacttctttactcccattcagcataagaaaaatgaaaccaaacggaattcttctcttttttagggggaaattccttaattgcttgttgaatatagattcatgtcgttattctatttttaataatgatgaaaatcaatatagtcaaagttaatacttatgtcatttggtttgcggacaagttatattggaactatataatacgtctattatagaatagtgattatttagaggatatacattttttttggataaatatttgatttattggattaaaaatagaatatacaggtaaggtctaaaacgtgtgtttgcttttacactaaataaacttgacctcgtacaattctaagaaaatatttgaaataaatgaattattttattgttaatcaattaaaaaaatcatagtatagatgagatgtgtgcatacttgacaataactatactaactaaaacaaggtatgtgaataattgatattccttttttaattattcttttttccagagtttggtcttggatgcagcagacacagttgctcttcacataaattggggaatggcattattgataaacaatcaaaaggccttgacgaaagcacaagaagagatagacacaaaagttggtaaggacagatgggtagaagagagtgatattaaggatttggtatacctccaagctattgttaaagaagtgttacgattatatccaccaggacctttgttagtaccacacgaaaatgtagaagattgtgttgttagtggatatcacattcctaaagggacaagattattcgcaaacgtcatgaaactgcaacgtgatcctaaactctggtctgatcctgatactttcgatccagagagattcattgctactgatattgactttcgtggtcagtactataagtatatcccgtttggttctggaagacgatcttgtccagggatgacttatgcattgcaagtggaacacttaacaatggcacatttgatccaaggtttcaattacagaactccaaatgacgagcccttggatatgaaggaaggtgcaggcataactatacgtaaggtaaatcctgtggaactgataatagcgcctcgcctggcacctgagctttattaaaacctaagatctttcatcttggttgatcattgtataatactcctaaatggatattcatttaccttttatcaattaattgtcagtacgagtttttctaatttggtacatttgtaataataagtaaagaataattgtgctaatatataa

SEQ ID NO: 40 - DNA, 2685 bp, Nicotiana tabacum
  5'UTR (1)...(30): CYP82E5v2 5' UTR
  exon (31)...(969): CYP82E5v2 exon 1 sequence
  intron (970)...(2023): CYP82E5v2 intron sequence
  exon (2024)...(2635): CYP82E5v2 exon 2 sequence
  3'UTR (2636)...(2685): CYP82E5v2 3' UTR
gattcccaagttcttttctaaaactccataatggtttctcccgtagaagccattgtaggactagtaacccttacacttctcttctacttcctatggcccaaaaaatttcaaataccttcaaaaccattaccaccgaaaattcccggagggtggccggtaatcggccatcttttctacttcgatgatgacggcgacgaccgtccattagctcgaaaactcggagacttagctgacaaatacggcccggttttcactttccggctaggccttccgcttgtgttagttgtaagcagttacgaagctgtaaaagactgcttctctacaaatgacgccattttctccaatcgtccagcttttctttacggtgaataccttggctacagtaatgccatgctatttttgacaaaatacggaccttattggcgaaaaaatagaaaattagtcattcaggaagttctctctgctagtcgtctcgaaaaattgaagcacgtgagatttggtaaaattcaaacgagcattaagagtttatacactcgaattgatggaaattcgagtacgataaatctaactgattggttagaagaattgaattttggtctgatcgtgaaaatgatcgctgggaaaaattatgaatccggtaaaggagatgaacaagtggagagatttaggaaagcgtttaaggattttataattttatcaatggagtttgtgttatgggatgcttttccaattccattgttcaaatgggtggattttcaaggccatgttaaggccatgaaaaggacatttaaggatatagattctgtttttcagaattggttagaggaacatgtcaagaaaagagaaaaaatggaggttaatgcacaagggaatgaacaagatttcattgatgtggtgctttcaaaaatgagtaatgaatatcttgatgaaggttactctcgtgatactgtcataaaagcaacagtgtttgtaagttcattttcatttttcattattcagtctgattttgaggaatagacaggttaataataatttaagtaattagattatctaaatactaaggatgattatatatagtaaaaatgtagaatgataaatggaaaaaagatgagaattttttgtgcctcgactaatctatatatctttgggagttaaaagtgcttcaccaaaggggacttttcctcatagctcaagttagaagtttgattatagatgaaagagtatttatcacttcacgaactctgatgataaaagtaaatgagatataaccagttataattgatagaataaaacttcattactcccattgagcataaaaaaaaaagtaaaagggacttcttctcttttttttagggagaaattctttaattgtttgttaaatatagattcatgttttttttttcttctatttctaataataatggttcttgaatcaggtcgttgactttgtagcagcaatatagtcaaagctaatatccatgttatttggttttcgaacaagttatactgaaattatatatacgggtattaaataataacattattatttataggatatactttttttattgggtaaatattacaacaacaacaactgactcagtaaaattttactagtggggtatggggagggtagtgtgtatgcagaccttacccctaccccgaaggagtagagggattgtttccgaaagaccctcggctcaagaaaacaaaaagagacaatatcagtaccaccacagatcatattattaggtaaatgttattttattgaattaaagatgaaatatacaggtaaggtataaaacgtgtatttgattttacactagataaatttgacctcgtacatctctaagagaaagctgaaataaatgaattttaaatttaaaaaaaaaattcattagtataatgagatgtgcatacttgacaattactatactaaatagaacaaggttcggcagatagtgacactaacctacttttgtattgaattatcctttttaattttattctaatttgtctacagagtttggtcttggatgctgcggacacagttgctcttcacatgaattggggaatggcattactgataaacaatcaacatgccttgaagaaagcacaagaagagatcgataaaaaagttggtaaggaaagatgggtagaagagagtgatattaaggatttggtctacctccaagctattgttaaagaagtgttacgattatatccaccaggacctttattagtacctcatgaaaatgtagaggattgtgttgttagtggatatcacattcctaaagggactagactattcgcgaacgttatgaaattgcagcgcgatcctaaactctggtcaaatcctgataagtttgatccagagagattcttcgctgatgatattgactaccgtggtcagcactatgagtttatcccatttggttctggaagacgatcttgtccggggatgacttatgcattacaagtggaacacctaacaatagcacatttgatccagggtttcaattacaaaactccaaatgacgagcccttggatatgaaggaaggtgcaggattaactatacgtaaagtaaatcctgtagaagtgacaattacggctcgcctggcacctgagctttattaaaaccttagatgttttatcttgattgtactaatatatatagcagaaaa